European Patent Application EP 4 644 571 A1, published November 5, 2025. Title: Method for detection of lung cancer using lung cancer-specific methylation marker gene. Applicant: GENOMICTREE, INC. The sequence listing filed with the application follows.

SEQUENCE LISTING (14 sequences)

SEQ ID NO: 1 - DNA, 1600 bp, synthetic construct
  misc_feature 1..1600: note = Synthetic Sequence
  source 1..1600: mol_type = other DNA
gtgtaaatgaggatagagagtgcgaaaggagggagaggcgaggagctgctctatttctagggaggttttggggagactgatcagctccaaggacagaccgctgggaagggaaaaacggcccacatcgaactggatgccggatggaaacctctctgcgctattagactgcgtccagtacagcagatggcacgagcacgtgcggcgctcagcttaggctctcggaggcagctgagttggaaatcccgacggaaagcacccacaagctcccactctgcgctggcccacccgcgtgcacgcccaccccccacgcgcgtccctggctcagaagcgcacagatgtttactgcttagagccggtaccgctggggagatcgagcgacttgcgcggcgcacagtgcggcgctggcagggctctgggctcccggtcgggggttcgagcggccaagggatgggggtgggggcggggagagtggggggagggcgaaagaccgccgagaggaggggggagtgggtggactaatgatgaaaaagtctcctccatcccagttccttaattaaatgcatggaaagaaccgaggcgagcacatctggtttcaatctacagccctttgatggcatcaaatgttcttttcccagatcagggctggaagttctgggctaactatggccgtttggagcccagaaaccatttacacacactcgtacccttctttctctccagtcgagcctcttgactataggacgaaaaaaaaaaaaagtctagcaatcaagggagtgcgggagtacggatgcgtgtgtgtgtgtgtgagtgcgcgtttaaagaacataaaacgccacaaataagcacttaatattttactgagtcgtcatacagtaactcatttctaatgagactgttaaagctgttaccaaattccaacaggtcatgaaaaaactgctcagcacctctctgtcttctgtcaggttagggctccgcagacggacgacagaggattatccgtagacttagatgggggttcctccgcccctctctgtcctcctgccaccacagccaggctggacgcagaaccgcacggaagcctccccaactcctgcctctgggagtgctcctgcctgcttcaaggaatctgggcagcgggaccctctgggtttagcgtcctcgcctggggaagcaactttggccttaccgtagaagttacaaaattggcgggggtagggagaaagattataatatatatttggagtcctttcttccagtttaataaacacgtacttttctcattgccctagtcctggtatgcctaatggcggggaaagcctcaaataaactcggtgccctctggatctccccaacctgcctttagtccttgcgagaggcgtgagagaacttcctattatcatcccttttgttatttttattacattatttaataggctccctctacggaaccaaaaatagccttaatatgcttactttctccctgtactccgccccaaactgttagaacagcagaaaatttttttttgggggggggcggtttgggggaaggcagaaggagaagaaaatttgattgtgatggtggtggattttttccaaattt

SEQ ID NO: 2 - DNA, 500 bp, synthetic construct
  misc_feature 1..500: note = Synthetic Sequence
  source 1..500: mol_type = other DNA
ccatgggaatcagcgtctcactttaggggacggtgggcaagggtcgcccttcgatagcgcggcggctggtccaccagagaaaccaagttttctaggtcgccggggaaaagcggaaaattagacttgagccagccttgctcctgtgagacattcgtgcactcataacccagcagtgggtgcctctacctagaatgagcccttcatttcccggatccgttcagggggaaacagcgaaatccccaaatccgcttccttacgtggctaataaaggggtgcttacagagcatggaaaaacaaaacaaagaaacaagaataccttgagtgttttgacgtttgaaaacccgactccggagaatcatggaatcatattccaagtttcagtgtctaatgaagtttaaggggacgcctattacttgggtttgtaaaatcgcggcgtcgcgcccgccccaagtcaaagctgagcagagcagggatggggaaggtctccggccccaggcgcg

SEQ ID NO: 3 - DNA, 24 bp, synthetic construct
  misc_feature 1..24: note = Synthetic Sequence
  source 1..24: mol_type = other DNA
tggggagattgattagttttaagg

SEQ ID NO: 4 - DNA, 23 bp, synthetic construct
  misc_feature 1..23: note = Synthetic Sequence
  source 1..23: mol_type = other DNA
aaatttccaactcaactacctcc

SEQ ID NO: 5 - DNA, 27 bp, synthetic construct
  misc_feature 1..27: note = Synthetic Sequence
  source 1..27: mol_type = other DNA
gtgggtgtttttatttagaatgagttt

SEQ ID NO: 6 - DNA, 25 bp, synthetic construct
  misc_feature 1..25: note = Synthetic Sequence
  source 1..25: mol_type = other DNA
actctataaacacccctttattaac

SEQ ID NO: 7 - DNA, 19 bp, synthetic construct
  misc_feature 1..19: note = Synthetic Sequence
  source 1..19: mol_type = other DNA
tttagtatagtagatggta

SEQ ID NO: 8 - DNA, 19 bp, synthetic construct
  misc_feature 1..19: note = Synthetic Sequence
  source 1..19: mol_type = other DNA
agaatgagttttttatttt

SEQ ID NO: 9 - DNA, 23 bp, synthetic construct
  misc_feature 1..23: note = Synthetic Sequence
  source 1..23: mol_type = other DNA
cggtttatatcgaattggatgtc

SEQ ID NO: 10 - DNA, 46 bp, synthetic construct
  misc_feature 1..46: note = Synthetic Sequence
  source 1..46: mol_type = other DNA
aaagattcggcgaccaccgacgaaaacctaaactaaacgccgcacg

SEQ ID NO: 11 - DNA, 18 bp, synthetic construct
  misc_feature 1..18: note = Synthetic Sequence
  source 1..18: mol_type = other DNA
gacggtgggtaagggtcg

SEQ ID NO: 12 - DNA, 49 bp, synthetic construct
  misc_feature 1..49: note = Synthetic Sequence
  source 1..49: mol_type = other DNA
aaagattcggcgaccaccgactaattttccgcttttccccgacgaccta

SEQ ID NO: 13 - DNA, 31 bp, synthetic construct
  misc_feature 1..31: note = Synthetic Sequence
  source 1..31: mol_type = other DNA
cgttattagattgcgtttagtatagtagatg

SEQ ID NO: 14 - DNA, 19 bp, synthetic construct
  misc_feature 1..19: note = Synthetic Sequence
  source 1..19: mol_type = other DNA
cgatagcgcggcggttggt